European Patent Application EP 4 234 579 A1, published August 30, 2023. Title: ANTI-CD73 ANTIBODY AND USE THEREOF. Applicant: Akeso Biopharma, Inc. AKESO PHARMACEUTICALS, INC. The sequence listing filed with the application follows.

SEQUENCE LISTING (36 sequences)

SEQ ID NO: 1 - DNA, 363 bp, Artificial sequence
  Nucleic acid sequence of the heavy chain variable region of 19F3
gaggtgcagctgcagcagtccggaccagagctggtgaagcctggcgcctccatgcggatgtcttgtaaggcctctggctacagcttcaccggctatacaatgaactgggtgaagcagtctcacggcaagaatctggagtggatcggcctgatcaacccttacaatgccggcaccagctataaccagaagtttaagggcaaggccaccctgacagtggacaagagctcctctaccgcctacatggagctgctgtccctgacatctgaggatagcgccgtgtactattgcgcccggtccgagtacagatatggcggcgactactttgattattggggccagggcaccacactgacagtgagctcc

SEQ ID NO: 2 - protein, 121 aa, Artificial sequence
  Amino acid sequence of the heavy chain variable region of 19F3
EVQLQQSGPELVKPGASMRMSCKASGYSFTGYTMNWVKQSHGKNLEWIGLINPYNAGTSYNQKFKGKATLTVDKSSSTAYMELLSLTSEDSAVYYCARSEYRYGGDYFDYWGQGTTLTVSS

SEQ ID NO: 3 - DNA, 339 bp, Artificial sequence
  Nucleic acid sequence of the light chain variable region of 19F3
gacatcgtgatgacccagtctccaagctccctggcaatgagcgtgggacagaaggtgacaatgtcttgtaagtctagccagagcctgctgaactcctctaatcagaagaactacctggcctggtatcagcagaagccaggccagtctcccaagctgctggtgtactttgccagcaccagggagtccggagtgcctgacagattcatcggctccggctctggcacagacttcaccctgacaatcagctccgtgcaggcagaggacctggcagattatttctgccagcagcactacgacaccccttatacatttggcggcggcaccaagctggagatcaag

SEQ ID NO: 4 - protein, 113 aa, Artificial sequence
  Amino acid sequence of the light chain variable region of 19F3
DIVMTQSPSSLAMSVGQKVTMSCKSSQSLLNSSNQKNYLAWYQQKPGQSPKLLVYFASTRESGVPDRFIGSGSGTDFTLTISSVQAEDLADYFCQQHYDTPYTFGGGTKLEIK

SEQ ID NO: 5 - DNA, 363 bp, Artificial sequence
  Nucleic acid sequence of the heavy chain variable region of 19F3H1L1(hG1DM)
caggtgcagctgcagcagtctggagcagaggtggtgaagccaggagcctctatgaagatgagctgtaaggccagcggctactccttcaccggctatacaatgaactgggtgaagcaggcccacggccagaatctggagtggatcggcctgatcaacccttacaatgccggcacctcttataaccagaagtttcagggcaaggccaccctgacagtggacaagtccacctctacagcctacatggagctgagctccctgcggagcgaggatacagccgtgtactattgcgcccggtccgagtacagatatggcggcgactactttgattattggggccagggcaccacactgaccgtgtctagc

SEQ ID NO: 6 - protein, 121 aa, Artificial sequence
  Amino acid sequence of the heavy chain variable region of 19F3H1L1(hG1DM)
QVQLQQSGAEVVKPGASMKMSCKASGYSFTGYTMNWVKQAHGQNLEWIGLINPYNAGTSYNQKFQGKATLTVDKSTSTAYMELSSLRSEDTAVYYCARSEYRYGGDYFDYWGQGTTLTVSS

SEQ ID NO: 7 - DNA, 339 bp, Artificial sequence
  Nucleic acid sequence of the light chain variable region of 19F3H1L1(hG1DM)
gacatcgtgatgacccagtccccaagctccctggcaatgtctgtgggagagagggtgacaatgtcctgtaagtctagccagtctctgctgaactcctctaatcagaagaactacctggcctggtatcagcagaagcccggccaggcccctaagctgctggtgtactttgcctctaccagggagagcggagtgccagacagattctctggcagcggctccggcacagacttcaccctgacaatcagctccgtgcaggcagaggacctggcagattatttctgccagcagcactacgataccccctatacatttggcggcggcaccaagctggagatcaag

SEQ ID NO: 8 - protein, 113 aa, Artificial sequence
  Amino acid sequence of the light chain variable region of 19F3H1L1(hG1DM)
DIVMTQSPSSLAMSVGERVTMSCKSSQSLLNSSNQKNYLAWYQQKPGQAPKLLVYFASTRESGVPDRFSGSGSGTDFTLTISSVQAEDLADYFCQQHYDTPYTFGGGTKLEIK

SEQ ID NO: 9 - DNA, 363 bp, Artificial sequence
  Nucleic acid sequence of the heavy chain variable region of 19F3H2L2(hG1DM) or 19F3H2L3(hG1DM)
caggtgcagctggtgcagtctggagcagaggtggtgaagccaggagcctctgtgaaggtgagctgtaaggccagcggctactccttcaccggctatacaatgaactgggtgaggcaggcaccaggacagaatctggagtggatcggcctgatcaacccttacaatgccggcacctcttataaccagaagtttcagggcaaggtgaccctgacagtggacaagtccacctctacagcctacatggagctgagctccctgcggagcgaggatacagccgtgtactattgcgcccggtccgagtacagatatggcggcgactactttgattattggggccagggcaccacactgaccgtgtctagc

SEQ ID NO: 10 - protein, 121 aa, Artificial sequence
  Amino acid sequence of the heavy chain variable region of 19F3H2L2(hG1DM) or 19F3H2L3(hG1DM)
QVQLVQSGAEVVKPGASVKVSCKASGYSFTGYTMNWVRQAPGQNLEWIGLINPYNAGTSYNQKFQGKVTLTVDKSTSTAYMELSSLRSEDTAVYYCARSEYRYGGDYFDYWGQGTTLTVSS

SEQ ID NO: 11 - DNA, 339 bp, Artificial sequence
  Nucleic acid sequence of the light chain variable region of 19F3H2L2(hG1DM)
gacatcgtgatgacccagtccccaagctccctggccgtgtctgtgggagagcgggtgacaatctcctgtaagtctagccagtctctgctgaactcctctaatcagaagaactacctggcctggtatcagcagaagcccggccaggcccctaagctgctgatctacttcgcctctaccagggagagcggagtgccagacagattctctggcagcggctccggcacagacttcaccctgacaatcagctccgtgcaggcagaggacgtggcagattactattgccagcagcactacgataccccctatacatttggcggcggcaccaagctggagatcaag

SEQ ID NO: 12 - protein, 113 aa, Artificial sequence
  Amino acid sequence of the light chain variable region of 19F3H2L2(hG1DM)
DIVMTQSPSSLAVSVGERVTISCKSSQSLLNSSNQKNYLAWYQQKPGQAPKLLIYFASTRESGVPDRFSGSGSGTDFTLTISSVQAEDVADYYCQQHYDTPYTFGGGTKLEIK

SEQ ID NO: 13 - DNA, 339 bp, Artificial sequence
  Nucleic acid sequence of the light chain variable region of 19F3H2L3(hG1DM)
gacatcgtgatgacccagtccccaagctccctggccgtgtctgtgggagagcgggtgacaatctcctgtaagtctagccagtctctgctgaactcctctaatcagaagaactacctggcctggtatcagcagaagcccggccaggcccctaagctgctgatctacttcgcctctaccagggagagcggagtgccagacagattctctggcagcggctccggcacagacttcaccctgacaatcagctccctgcaggcagaggacgtggccgtgtactattgccagcagcactacgataccccctatacatttggcggcggcaccaagctggagatcaag

SEQ ID NO: 14 - protein, 113 aa, Artificial sequence
  Amino acid sequence of the light chain variable region of 19F3H2L3(hG1DM)
DIVMTQSPSSLAVSVGERVTISCKSSQSLLNSSNQKNYLAWYQQKPGQAPKLLIYFASTRESGVPDRFSGSGSGTDFTLTISSLQAEDVAVYYCQQHYDTPYTFGGGTKLEIK

SEQ ID NO: 15 - protein, 8 aa, Artificial sequence
  Amino acid sequence of HCDR1 of 19F3, 19F3H1L1(hG1DM),19F3H2L2 (hG1DM)or 19F3H2L3(hG1DM)
GYSFTGYT

SEQ ID NO: 16 - protein, 8 aa, Artificial sequence
  Amino acid sequence of HCDR2 of 19F3, 19F3H1L1(hG1DM), 19F3H2L2 (hG1DM) or19F3H2L3(hG1DM)
INPYNAGT

SEQ ID NO: 17 - protein, 14 aa, Artificial sequence
  Amino acid sequence of HCDR3 of 19F3, 19F3H1L1(hG1DM), 19F3H2L2 (hG1DM) or 19F3H2L3(hG1DM)
ARSEYRYGGDYFDY

SEQ ID NO: 18 - protein, 12 aa, Artificial sequence
  Amino acid sequence of LCDR1 of 19F3, 19F3H1L1(hG1DM), 19F3H2L2 (hG1DM) or 19F3H2L3(hG1DM)
QSLLNSSNQKNY

SEQ ID NO: 19 - protein, 3 aa, Artificial sequence
  Amino acid sequence of LCDR2 of 19F3, 19F3H1L1(hG1DM), 19F3H2L2 (hG1DM) or 19F3H2L3(hG1DM)
FAS

SEQ ID NO: 20 - protein, 9 aa, Artificial sequence
  Amino acid sequence of LCDR3 of 19F3, 19F3H1L1(hG1DM), 19F3H2L2 (hG1DM) or 19F3H2L3(hG1DM)
QQHYDTPYT

SEQ ID NO: 21 - protein, 330 aa, Artificial sequence
  Sequence of the heavy chain constant region of 19F3H1L1(hG1DM), 19F3H2L2(hG1DM) or 19F3H2L3(hG1DM)
ASTKGPSVFPLAPSSKSTSGGTAALGCLVKDYFPEPVTVSWNSGALTSGVHTFPAVLQSSGLYSLSSVVTVPSSSLGTQTYICNVNHKPSNTKVDKKVEPKSCDKTHTCPPCPAPEAAGGPSVFLFPPKPKDTLMISRTPEVTCVVVDVSHEDPEVKFNWYVDGVEVHNAKTKPREEQYNSTYRVVSVLTVLHQDWLNGKEYKCKVSNKALPAPIEKTISKAKGQPREPQVYTLPPSRDELTKNQVSLTCLVKGFYPSDIAVEWESNGQPENNYKTTPPVLDSDGSFFLYSKLTVDKSRWQQGNVFSCSVMHEALHNHYTQKSLSLSPGK

SEQ ID NO: 22 - protein, 107 aa, Artificial sequence [sequence omitted]

SEQ ID NO: 23 - protein, 8 aa, Artificial sequence
  Amino acid sequence of HCDR1 involved in the heavy chain variable region of BiAb004 (hG1TM)
GFAFSSYD

SEQ ID NO: 24 - protein, 8 aa, Artificial sequence
  Amino acid sequence of HCDR2 involved in the heavy chainvariable region of BiAb004 (hG1TM)
ISGGGRYT

SEQ ID NO: 25 - protein, 11 aa, Artificial sequence
  Amino acid sequence of HCDR3 involved in the heavy chain variable region of BiAb004 (hG1TM)
ANRYGEAWFAY

SEQ ID NO: 26 - protein, 8 aa, Artificial sequence
  Amino acid sequence of HCDR4 involved in the heavy chain variable region of BiAb004 (hG1TM)
GYSFTGYT

SEQ ID NO: 27 - protein, 8 aa, Artificial sequence
  Amino acid sequence of HCDR5 involved in the heavy chain variable region of BiAb004 (hG1TM)
INPYNNIT

SEQ ID NO: 28 - protein, 8 aa, Artificial sequence
  Amino acid sequence of HCDR6 involved in the heavy chain variable region of BiAb004 (hG1TM)
ARLDYRSY

SEQ ID NO: 29 - protein, 9 aa, Artificial sequence
  Amino acid sequence of HCDR7 involved in the heavy chain variable region of BiAb004 (hG1TM)
TGAVTTSNF

SEQ ID NO: 30 - protein, 3 aa, Artificial sequence
  Amino acid sequence of HCDR8 involved in the heavy chain variable region of BiAb004 (hG1TM)
GTN

SEQ ID NO: 31 - protein, 9 aa, Artificial sequence
  Amino acid sequence of HCDR9 involved in the heavy chain variable region of BiAb004 (hG1TM)
ALWYSNHWV

SEQ ID NO: 32 - protein, 6 aa, Artificial sequence
  Amino acid sequence of LCDR1 involved in the heavy chain variable region of BiAb004 (hG1TM)
QDINTY

SEQ ID NO: 33 - protein, 3 aa, Artificial sequence
  Amino acid sequence of LCDR2 involved in the heavy chain variable region of BiAb004 (hG1TM)
RAN

SEQ ID NO: 34 - protein, 9 aa, Artificial sequence
  Amino acid sequence of LCDR3 involved in the heavy chain variable region of BiAb004 (hG1TM)
LQYDEFPLT

SEQ ID NO: 35 - protein, 713 aa, Artificial sequence
  Amino acid sequence of the heavy chain of BiAb004(hG1TM)
EVQLVESGGGLVQPGGSLRLSCAASGFAFSSYDMSWVRQAPGKGLDWVATISGGGRYTYYPDSVKGRFTISRDNSKNNLYLQMNSLRAEDTALYYCANRYGEAWFAYWGQGTLVTVSSASTKGPSVFPLAPSSKSTSGGTAALGCLVKDYFPEPVTVSWNSGALTSGVHTFPAVLQSSGLYSLSSVVTVPSSSLGTQTYICNVNHKPSNTKVDKKVEPKSCDKTHTCPPCPAPEAAGAPSVFLFPPKPKDTLMISRTPEVTCVVVDVSHEDPEVKFNWYVDGVEVHNAKTKPREEQYNSTYRVVSVLTVLHQDWLNGKEYKCKVSNKALPAPIEKTISKAKGQPREPQVYTLPPSRDELTKNQVSLTCLVKGFYPSDIAVEWESNGQPENNYKTTPPVLDSDGSFFLYSKLTVDKSRWQQGNVFSCSVMHEALHNHYTQKSLSLSPGKGGGGSGGGGSGGGGSGGGGSQVQLVESGAEVKKPGASVKVSCKASGYSFTGYTMNWVRQAPGQCLEWIGLINPYNNITNYAQKFQGRVTFTVDTSISTAYMELSRLRSDDTGVYFCARLDYRSYWGQGTLVTVSAGGGGSGGGGSGGGGSGGGGSQAVVTQEPSLTVSPGGTVTLTCGSSTGAVTTSNFPNWVQQKPGQAPRSLIGGTNNKASWTPARFSGSLLGGKAALTISGAQPEDEAEYYCALWYSNHWVFGCGTKLTVLR

SEQ ID NO: 36 - protein, 214 aa, Artificial sequence
  Amino acid sequence of the light chain of BiAb004(hG1TM)
DIQMTQSPSSMSASVGDRVTFTCRASQDINTYLSWFQQKPGKSPKTLIYRANRLVSGVPSRFSGSGSGQDYTLTISSLQPEDMATYYCLQYDEFPLTFGAGTKLELKRTVAAPSVFIFPPSDEQLKSGTASVVCLLNNFYPREAKVQWKVDNALQSGNSQESVTEQDSKDSTYSLSSTLTLSKADYEKHKVYACEVTHQGLSSPVTKSFNRGEC